European Patent Application EP 4 692 800 A2, published February 11, 2026. Title: METHODS AND KITS FOR DETECTING ADENO-ASSOCIATED VIRUSES. Applicant: LONZA HOUSTON, INC. The sequence listing filed with the application follows.

SEQUENCE LISTING (2 sequences)

SEQ ID NO: 1 - protein, 6 aa, synthetic construct
LQSANT

SEQ ID NO: 2 - protein, 6 aa, synthetic construct
LQQQNT